European Patent Application EP 4 501 350 A1, published February 5, 2025. Title: Anti-Netrin-4 antibody and utilization thereof. Applicant: 大阪大学. The sequence listing filed with the application follows.

SEQUENCE LISTING (14 sequences)

SEQ ID NO: 1 - protein, 628 aa, Homo sapiens
MGSCARLLLLWGCTVVAAGLSGVAGVSSRCEKACNPRMGNLALGRKLWADTTCGQNATELYCFYSENTDLTCRQPKCDKCNAAYPHLAHLPSAMADSSFRFPRTWWQSAEDVHREKIQLDLEAEFYFTHLIVMFKSPRPAAMVLDRSQDFGKTWKPYKYFATNCSATFGLEDDVVKKGAICTSKYSSPFPCTGGEVIFKALSPPYDTENPYSAKVQEQLKITNLRVQLLKRQSCPCQRNDLNEEPQHFTHYAIYDFIVKGSCFCNGHADQCIPVHGFRPVKAPGTFHMVHGKCMCKHNTAGSHCQHCAPLYNDRPWEAADGKTGAPNECRTCKCNGHADTCHFDVNVWEASGNRSGGVCDDCQHNTEGQYCQRCKPGFYRDLRRPFSAPDACKPCSCHPVGSAVLPANSVTFCDPSNGDCPCKPGVAGRRCDRCMVGYWGFGDYGCRPCDCAGSCDPITGDCISSHTDIDWYHEVPDFRPVHNKSEPAWEWEDAQGFSALLHSGKCECKEQTLGNAKAFCGMKYSYVLKIKILSAHDKGTHVEVNVKIKKVLKSTKLKIFRGKRTLYPESWTDRGCTCPILNPGLEYLVAGHEDIRTGKLIVNMKSFVQHWKPSLGRKVMDILKRECK

SEQ ID NO: 2 - protein, 11 aa, Homo sapiens
TGGEVIFKALS

SEQ ID NO: 3 - protein, 444 aa, Mus musculus
QVQLHQSGPELVRPGASVTLSCKASGYTFTDYEMHWVKQTPVHGLEWIGAIDPETGDTVYNQKFKGKATLTADKSSSTAYMELSSLTSEDSAVYYCVDGFSDHYWGQGTTLTVSSAKTTAPSVYPLAPVCGDTTGSSVTLGCLVKGYFPEPVTLTWNSGSLSSGVHTFPAVLQSDLYTLSSSVTVTSSTWPSQSITCNVAHPASSTKVDKKIEPRGSPTHKPCPPCPAPNLLGGPSVFIFPPKIKDVLMISLSPMVTCVVVDVSEDDPDVHVSWFVNNVEVHTAQTQTHREDYNSTIRVVSALPIQHQDWMSGKEFKCKVNNKALPAPIERTISKPKGPVRAPQVYVLPPPEEEMTKKQVTLTCMITDFMPEDIYVEWTNNGQTELNYKNTEPVLDSDGSYFMYSKLRVEKKNWVERNSYSCSVVHEGLHNHHTTKSFSRTPGK

SEQ ID NO: 4 - protein, 219 aa, Mus musculus
VLVLTQTPLSLPVRLGDRASISCRSSQSLVHSSGNTFLHWYLQKPGQSPKLLIYKVSSRFSGVPDRFSGSGSGTDFTLKISRMEAEDLGVYFCSQSTHIPYTFGGGTKLEIKRADAAPTVSIFPPSSEQLTSGGASVVCFLNNFYPKDINVKWKIDGSERQNGVLNSWTDQDSKDSTYSMSSTLTLTKDEYERHNSYTCEATHKTSTSPIVKSFNRNEC

SEQ ID NO: 5 - protein, 115 aa, Mus musculus
QVQLHQSGPELVRPGASVTLSCKASGYTFTDYEMHWVKQTPVHGLEWIGAIDPETGDTVYNQKFKGKATLTADKSSSTAYMELSSLTSEDSAVYYCVDGFSDHYWGQGTTLTVSS

SEQ ID NO: 6 - protein, 111 aa, Mus musculus
VLVLTQTPLSLPVRLGDRASISCRSSQSLVHSSGNTFLHWYLQKPGQSPKLLIYKVSSRFSGVPDRFSGSGSGTDFTLKISRMEAEDLGVYFCSQSTHIPYTFGGGTKLEI

SEQ ID NO: 7 - protein, 5 aa, Mus musculus
DYEMH

SEQ ID NO: 8 - protein, 17 aa, Mus musculus
AIDPETGDTVYNQKFKG

SEQ ID NO: 9 - protein, 6 aa, Mus musculus
GFSDHY

SEQ ID NO: 10 - protein, 16 aa, Mus musculus
RSSQSLVHSSGNTFLH

SEQ ID NO: 11 - protein, 7 aa, Mus musculus
KVSSRFS

SEQ ID NO: 12 - protein, 9 aa, Mus musculus
SQSTHIPYT

SEQ ID NO: 13 - DNA, 345 bp, Mus musculus
  source 1..345: mol_type = genomic DNA
caggttcaactgcaccagtctggacctgaactggtgaggcctggggcttcagtgacgctgtcctgcaaggcttcgggctacacatttactgactatgagatgcactgggtgaagcagacacctgtgcatggcctggagtggattggagctattgatcctgaaactggtgacactgtctacaatcagaaattcaagggcaaggccacactgactgcagacaaatcctccagcacagcctacatggagctcagcagcctgacatctgaggactctgccgtctattattgtgtcgatggtttttctgatcattactggggccaaggcaccactctcacagtttcctca

SEQ ID NO: 14 - DNA, 333 bp, Mus musculus
  source 1..333: mol_type = genomic DNA
gttcttgtgctgacccagactccactctccctgcctgtccgtcttggagatagagcctccatctcttgcagatccagtcagagccttgtacacagtagtggaaacacctttttacattggtacctgcagaagccaggccagtctccaaagctcctgatctacaaagtttccagtcgattttctggggtcccagacaggttcagtggcagtggatcagggacagatttcacactcaagatcagcagaatggaggctgaggatctgggagtttatttctgctctcaaagtacacatattccgtacacgttcggaggggggaccaagctggaaata